European Patent Specification EP 3 160 964 B1, published March 13, 2024. Title: Aryl Receptor Modulators and Methods of Making and Using the Same. Applicant: Nogra Pharma Limited. The sequence listing filed with the application follows.

SEQUENCE LISTING (10 sequences)

SEQ ID NO: 1 - DNA, 20 bp, Artificial Sequence
  Human IFN-gamma forward primer
tggagaccatcaaggaagac

SEQ ID NO: 2 - DNA, 20 bp, Artificial Sequence
  Human IFN-gamma reverse primer
gcgttggacattcaagtcag

SEQ ID NO: 3 - DNA, 27 bp, Artificial Sequence
  beta-actin forward primer
aagatgacccagatcatgtttgagacc

SEQ ID NO: 4 - DNA, 20 bp, Artificial Sequence
  beta-actin reverse primer
agccagtccagacgcaggat

SEQ ID NO: 5 - DNA, 20 bp, Artificial Sequence
  Human Col1A1 primer
ggacacagaggtttcagtgg

SEQ ID NO: 6 - DNA, 21 bp, Artificial Sequence
  Human Col3A1 primer
ggagaatgttgtgcagtttgc

SEQ ID NO: 7 - DNA, 20 bp, Artificial Sequence
  Human alpha-SMA primer
tctggagatggtgtcaccca

SEQ ID NO: 8 - DNA, 20 bp, Artificial Sequence
  human AhR forward primer
gagcacaaatcagagactgg

SEQ ID NO: 9 - DNA, 20 bp, Artificial Sequence
  Human AhR reverse primer
tggaggaagcatagaagacc

SEQ ID NO: 10 - DNA, 20 bp, Artificial Sequence
  mouse Col1A2 primer
acacagtggtatggatggac